European Patent Application EP 4 234 570 A2, published August 30, 2023. Title: PROGRAMMED CELL DEATH 1 (PD1) SPECIFIC NUCLEASES. Applicant: SANGAMO THERAPEUTICS, INC. The sequence listing filed with the application follows.

SEQUENCE LISTING (6 sequences)

SEQ ID NO: 1 - protein, 579 aa, unidentified
  REGION 1..579: note = Description of Unknown: FokI protein sequence
MVSKIRTFGWVQNPGKFENLKRVVQVFDRNSKVHNEVKNIKIPTLVKESKIQKELVAIMNQHDLIYTYKELVGTGTSIRSEAPCDAIIQATIADQGNKKGYIDNWSSDGFLRWAHALGFIEYINKSDSFVITDVGLAYSKSADGSAIEKEILIEAISSYPPAIRILTLLEDGQHLTKFDLGKNLGFSGESGFTSLPEGILLDTLANAMPKDKGEIRNNWEGSSDKYARMIGGWLDKLGLVKQGKKEFIIPTLGKPDNKEFISHAFKITGEGLKVLRRAKGSTKFTRVPKRVYWEMLATNLTDKEYVRTRRALILEILIKAGSLKIEQIQDNLKKLGFDEVIETIENDIKGLINTGIFIEIKGRFYQLKDHILQFVIPNRGVTKQLVKSELEEKKSELRHKLKYVPHEYIELIEIARNSTQDRILEMKVMEFFMKVYGYRGKHLGGSRKPDGAIYTVGSPIDYGVIVDTKAYSGGYNLPIGQADEMQRYVEENQTRNKHINPNEWWKVYPSSVTEFKFLFVSGHFKGNYKAQLTRLNHITNCNGAVLSVEELLIGGEMIKAGTLTLEEVRRKFNNGEINF

SEQ ID NO: 2 - DNA, 1155 bp, synthetic construct
  misc_feature 1..1155: note = Description of Artificial Sequence: Synthetic polynucleotide
  source 1..1155: mol_type = other DNA
atggactacaaagaccatgacggtgattataaagatcatgacatcgattacaaggatgacgatgacaagatggcccccaagaagaagaggaaggtgggcattcacggggtacccgccgctatggctgagaggcccttccagtgtcgaatctgcatgcgtaagtttgcccagtccggccacctgtcccgccataccaagatacacacgggcgagaagcccttccagtgtcgaatctgcatgcgtaacttcagtcgtagtgacagcctgagcgtacacatccgcacccacacaggcgagaagccttttgcctgtgacatttgtgggaggaaatttgcccacaacgacagccgcaaaaaccataccaagatacacacgggatctcagaagcccttccagtgtcgaatctgcatgcgtaacttcagtcgctccgacgacctgacccgccacatccgcacccacacaggcgagaagccttttgcctgtgacatttgtgggaggaagtttgcccgctccgaccacctgacccagcataccaagatacacctgcggggatcccagctggtgaagagcgagctggaggagaagaagtccgagctgcggcacaagctgaagtacgtgccccacgagtacatcgagctgatcgagatcgccaggaacagcacccaggaccgcatcctggagatgaaggtgatggagttcttcatgaaggtgtacggctacaggggaaagcacctgggcggaagcagaaagcctgacggcgccatctatacagtgggcagccccatcgattacggcgtgatcgtggacacaaaggcctacagcggcggctacaatctgcctatcggccaggccgacgagatgcagagatacgtggaggagaaccagacccggaataagcacatcaaccccaacgagtggtggaaggtgtaccctagcagcgtgaccgagttcaagttcctgttcgtgagcggccacttcaagggcaactacaaggcccagctgaccaggctgaaccacatcaccaactgcaatggcgccgtgctgagcgtggaggagctgctgatcggcggcgagatgatcaaagccggcaccctgacactggaggaggtgcggcgcaagttcaacaacggcgagatcaacttcagatcttgataa

SEQ ID NO: 3 - protein, 383 aa, synthetic construct
  REGION 1..383: note = Description of Artificial Sequence: Synthetic polypeptide
MDYKDHDGDYKDHDIDYKDDDDKMAPKKKRKVGIHGVPAAMAERPFQCRICMRKFAQSGHLSRHTKIHTGEKPFQCRICMRNFSRSDSLSVHIRTHTGEKPFACDICGRKFAHNDSRKNHTKIHTGSQKPFQCRICMRNFSRSDDLTRHIRTHTGEKPFACDICGRKFARSDHLTQHTKIHLRGSQLVKSELEEKKSELRHKLKYVPHEYIELIEIARNSTQDRILEMKVMEFFMKVYGYRGKHLGGSRKPDGAIYTVGSPIDYGVIVDTKAYSGGYNLPIGQADEMQRYVEENQTRNKHINPNEWWKVYPSSVTEFKFLFVSGHFKGNYKAQLTRLNHITNCNGAVLSVEELLIGGEMIKAGTLTLEEVRRKFNNGEINFRS

SEQ ID NO: 4 - DNA, 1155 bp, synthetic construct
  misc_feature 1..1155: note = Description of Artificial Sequence: Synthetic polynucleotide
  source 1..1155: mol_type = other DNA
atggactacaaagaccatgacggtgattataaagatcatgacatcgattacaaggatgacgatgacaagatggcccccaagaagaagaggaaggtgggcattcacggggtacccgccgctatggctgagaggcccttccagtgtcgaatctgcatgtgtaagtttgcccgcaacgccgccctgacccgccataccaagatacacacgggcgagaagccgttccagtgtcgcatctgcatgcgtaacttcagtcgctccgacgagctgacccgccacatccgcacccacacaggcgagaagccttttgcttgcgacatttgtgggaggaagtttgcccggcaccaccacctggccgcccataccaagatacacacgggatctcagaagcccttccagtgtcgaatctgcatgcgtaacttcagtacccgcccggtgctgaagcgccacatccgcacccacacaggcgagaagccttttgcttgcgacatttgtgggaggaagtttgccgaccgctccgccctggcccgccataccaagatacacctgcggggatcccagctggtgaagagcgagctggaggagaagaagtccgagctgcggcacaagctgaagtacgtgccccacgagtacatcgagctgatcgagatcgccaggaacagcacccaggaccgcatcctggagatgaaggtgatggagttcttcatgaaggtgtacggctacaggggaaagcacctgggcggaagcagaaagcctgacggcgccatctatacagtgggcagccccatcgattacggcgtgatcgtggacacaaaggcctacagcggcggctacaatctgcctatcggccaggccgacgagatgcagagatacgtggaggagaaccagacccggaataagcacatcaaccccaacgagtggtggaaggtgtaccctagcagcgtgaccgagttcaagttcctgttcgtgagcggccacttcaagggcaactacaaggcccagctgaccaggctgaaccacatcaccaactgcaatggcgccgtgctgagcgtggaggagctgctgatcggcggcgagatgatcaaagccggcaccctgacactggaggaggtgcggcgcaagttcaacaacggcgagatcaacttcagatcttgataa

SEQ ID NO: 5 - protein, 383 aa, synthetic construct
  REGION 1..383: note = Description of Artificial Sequence: Synthetic polypeptide
MDYKDHDGDYKDHDIDYKDDDDKMAPKKKRKVGIHGVPAAMAERPFQCRICMCKFARNAALTRHTKIHTGEKPFQCRICMRNFSRSDELTRHIRTHTGEKPFACDICGRKFARHHHLAAHTKIHTGSQKPFQCRICMRNFSTRPVLKRHIRTHTGEKPFACDICGRKFADRSALARHTKIHLRGSQLVKSELEEKKSELRHKLKYVPHEYIELIEIARNSTQDRILEMKVMEFFMKVYGYRGKHLGGSRKPDGAIYTVGSPIDYGVIVDTKAYSGGYNLPIGQADEMQRYVEENQTRNKHINPNEWWKVYPSSVTEFKFLFVSGHFKGNYKAQLTRLNHITNCNGAVLSVEELLIGGEMIKAGTLTLEEVRRKFNNGEINFRS

SEQ ID NO: 6 - protein, 9 aa, unidentified
  REGION 1..9: note = Description of Unknown: "LAGLIDADG" family peptide motif sequence
LAGLIDADG